European Patent Application EP 4 717 762 A1, published April 1, 2026. Title: Curcumin producing gram positive bacteria. Applicant: Universitaet des Saarlandes, eine Koerperschaft des Oeffentlichen Rechts. Application EP. The sequence listing filed with the application follows.

SEQUENCE LISTING (31 sequences)

SEQ ID NO: 1 - protein, 402 aa, Oryza sativa
  REGION 1..402: note = curcuminoid synthase (CUS)
MAPTTTMGSALYPLGEMRRSQRADGLAAVLAIGTANPPNCVTQEEFPDFYFRVTNSDHLTALKDKFKRICQEMGVQRRYLHHTEEMLSAHPEFVDRDAPSLDARLDIAADAVPELAAEAAKKAIAEWGRPAADITHLVVTTNSGAHVPGVDFRLVPLLGLRPSVRRTMLHLNGCFAGCAALRLAKDLAENSRGARVLVVAAELTLMYFTGPDEGCFRTLLVQGLFGDGAAAVIVGADADDVERPLFEIVSAAQTIIPESDHALNMRFTERRLDGVLGRQVPGLIGDNVERCLLDMFGPLLGGDGGGGWNDLFWAVHPGSSTIMDQVDAALGLEPGKLAASRRVLSDYGNMSGATVIFALDELRRQRKEAAAAGEWPELGVMMAFGPGMTVDAMLLHATSHVN

SEQ ID NO: 2 - protein, 402 aa, Oryza sativa; identical to SEQ ID NO: 1
  REGION 1..402: note = curcuminoid synthase (CUS) (codon-optimized)

SEQ ID NO: 3 - protein, 389 aa, Curcuma longa
  REGION 1..389: note = diketide-CoA synthase (DCS)
MEANGYRITHSADGPATILAIGTANPTNVVDQNAYPDFYFRVTNSEYLQELKAKFRRICEKAAIRKRHLYLTEEILRENPSLLAPMAPSFDARQAIVVEAVPKLAKEAAEKAIKEWGRPKSDITHLVFCSASGIDMPGSDLQLLKLLGLPPSVNRVMLYNVGCHAGGTALRVAKDLAENNRGARVLAVCSEVTVLSYRGPHPAHIESLFVQALFGDGAAALVVGSDPVDGVERPIFEIASASQVMLPESAEAVGGHLREIGLTFHLKSQLPSIIASNIEQSLTTACSPLGLSDWNQLFWAVHPGGRAILDQVEARLGLEKDRLAATRHVLSEYGNMQSATVLFILDEMRNRSAAEGHATTGEGLDWGVLLGFGPGLSIETVVLHSCRLN

SEQ ID NO: 4 - protein, 389 aa, Curcuma longa; identical to SEQ ID NO: 3
  REGION 1..389: note = diketide-CoA synthase (DCS) (codon-optimized)

SEQ ID NO: 5 - protein, 389 aa, Curcuma longa
  REGION 1..389: note = curcumin synthase 1 (CURS1)
MANLHALRREQRAQGPATIMAIGTATPPNLYEQSTFPDFYFRVTNSDDKQELKKKFRRMCEKTMVKKRYLHLTEEILKERPKLCSYKEASFDDRQDIVVEEIPRLAKEAAEKAIKEWGRPKSEITHLVFCSISGIDMPGADYRLATLLGLPLTVNRLMIYSQACHMGAAMLRIAKDLAENNRGARVLVVACEITVLSFRGPNEGDFEALAGQAGFGDGAGAVVVGADPLEGIEKPIYEIAAAMQETVAESQGAVGGHLRAFGWTFYFLNQLPAIIADNLGRSLERALAPLGVREWNDVFWVAHPGNWAIMDAIEAKLQLSPDKLSTARHVFTEYGNMQSATVYFVMDELRKRSAVEGRSTTGDGLQWGVLLGFGPGLSIETVVLRSMPL

SEQ ID NO: 6 - protein, 389 aa, Curcuma longa; identical to SEQ ID NO: 5
  REGION 1..389: note = curcumin synthase 1 (CURS1) (codon-optimized)

SEQ ID NO: 7 - protein, 391 aa, Curcuma longa
  REGION 1..391: note = curcumin synthase 2 (CURS2)
MAMISLQAMRKAQRAQGPATILAVGTANPPNLYEQDTYPDYYFRVTNSEHKQELKNKFRLMCEKTMVKRRYLYLTPEILKERPKLCSYMEPSFDDRQDIVVEEVPKLAAEAAENAIKEWGGDKSAITHLVFCSISGIDMPGADYRLAQLLGLPLAVNRLMLYSQACHMGAAMLRIAKDIAENNRSARVLVVACEITVLSFRGPDERDFQALAGQAGFGDGAGAMIVGADPVLGVERPLYHIMSATQTTVPESEKAVGGHLREVGLTFHFFNQLPAIIADNVGNSLAEAFEPIGIKDWNNIFWVAHPGNWAIMDAIETKLGLEQSKLATARHVFSEFGNMQSATVYFVMDELRKRSAAENRATTGDGLRWGVLFGFGPGISIETVVLQSVPL

SEQ ID NO: 8 - protein, 390 aa, Curcuma longa
  REGION 1..390: note = curcumin synthase 3 (CURS3)
MGSLQAMRRAQRAQGPATIMAVGTSNPPNLYEQTSYPDFYFRVTNSDHKHALKNKFRVICEKTKVKRRYLHLTEEILKQRPKLCSYMEPSFDDRQDIVVEEIPKLAKEAAEKAIKEWGRPKSEITHLVFCSISGIDMPGADYRLATLLGLPLSVNRLMLYSQACHMGAQMLRIAKDLAENNRGARVLAVSCEITVLSFRGPDAGDFEALACQAGFGDGAAAVVVGADPLPGVERPIYEIAAAMQETVPESERAVGGHLREIGWTFHFFNQLPKLIAENIEGSLARAFKPLGISEWNDVFWVAHPGNWGIMDAIETKLGLEQGKLATARHVFSEYGNMQSATVYFVMDEVRKRSAAEGRATTGEGLEWGVLFGFGPGLTIETVVLRSVPLP

SEQ ID NO: 9 - protein, 561 aa, Arabidopsis thaliana
  REGION 1..561: note = 4-coumarate-CoA ligase (4CL)
MAPQEQAVSQVMEKQSNNNNSDVIFRSKLPDIYIPNHLSLHDYIFQNISEFATKPCLINGPTGHVYTYSDVHVISRQIAANFHKLGVNQNDVVMLLLPNCPEFVLSFLAASFRGATATAANPFFTPAEIAKQAKASNTKLIITEARYVDKIKPLQNDDGVVIVCIDDNESVPIPEGCLRFTELTQSTTEASEVIDSVEISPDDVVALPYSSGTTGLPKGVMLTHKGLVTSVAQQVDGENPNLYFHSDDVILCVLPMFHIYALNSIMLCGLRVGAAILIMPKFEINLLLELIQRCKVTVAPMVPPIVLAIAKSSETEKYDLSSIRVVKSGAAPLGKELEDAVNAKFPNAKLGQGYGMTEAGPVLAMSLGFAKEPFPVKSGACGTVVRNAEMKIVDPDTGDSLSRNQPGEICIRGHQIMKGYLNNPAATAETIDKDGWLHTGDIGLIDDDDELFIVDRLKELIKYKGFQVAPAELEALLIGHPDITDVAVVAMKEEAAGEVPVAFVVKSKDSELSEDDVKQFVSKQVVFYKRINKVFFTESIPKAPSGKILRKDLRAKLANGL

SEQ ID NO: 10 - protein, 561 aa, Arabidopsis thaliana; identical to SEQ ID NO: 9
  REGION 1..561: note = 4-coumarate-CoA ligase (4CL) (codon-optimized)

SEQ ID NO: 11 - DNA, 1209 bp, Oryza sativa
  source 1..1209: mol_type = other DNA
atggcaccgacgacgaccatgggaagcgccttatacccgctcggcgaaatgcggcggtcgcagcgcgccgacgggctcgccgccgtgctcgccatcggcaccgccaaccctcccaactgcgttacccaggaggagttccccgacttctacttccgcgtcaccaacagcgaccacctcactgccctcaaggacaagttcaagcgtatctgtcaggaaatgggcgtgcagaggcggtacctgcaccacacggaggagatgctgtccgcacacccggagttcgtggaccgcgacgcgccgtcgctcgacgcgcggctggacatcgccgcggacgccgtgccggagctggcggcggaggccgccaagaaggcgatcgccgagtggggccgcccggccgccgacatcacccacctcgtcgtcaccaccaactccggcgcccacgtcccgggtgtcgacttccgcctcgtcccgctcctcggcctccgcccctccgtgcgccgcaccatgctccacctcaacggctgcttcgccggctgcgccgcgctccgcctcgccaaggacctcgccgagaacagccgcggcgcgcgcgtcctcgtcgtcgccgccgagctcaccctcatgtacttcaccgggcccgacgagggctgcttcaggacgctcctcgtccagggcctgttcggcgacggcgcggccgccgtcattgtcggcgccgacgccgacgacgtcgagcgcccgctgttcgagatagtgtcggcggcgcagacgatcatcccggagtcggaccacgccctgaacatgcggttcacggagcgccgcttggacggcgtcctcgggcggcaggtcccggggctcatcggggacaacgtcgagcggtgcctcctggacatgttcggcccacttctcggcggcgacggcggcggcgggtggaacgacctgttctgggcggtgcacccgggctcgtcgacgatcatggaccaggtcgacgcggcgctcggcctcgagcccggcaagctggcggcgagccgccgtgtgctcagcgactacgggaacatgtctggcgctacggtgatcttcgcgctggacgagctgcgccggcagcgcaaggaggcggcggcggcgggtgaatggccggagttgggagtgatgatggcgttcggcccggggatgaccgttgatgcgatgctgttgcacgccacctctcatgtgaattaa

SEQ ID NO: 12 - DNA, 1209 bp, synthetic construct
  source 1..1209: mol_type = other DNA
atggccccaaccaccaccatgggctccgcactgtacccactgggtgaaatgcgccgctcccagcgtgctgatggtctggcagctgtgctggctatcggtaccgccaacccaccaaactgcgtcacccaggaagagttcccagatttctacttccgcgttaccaactccgaccacctgaccgcactgaaggataagttcaagcgcatctgccaggaaatgggcgtgcagcgccgctacctgcaccacaccgaagagatgctgtccgctcacccagagttcgttgatcgtgatgcaccatccctggatgcacgtctggacatcgccgcagatgcagtgccagaactggctgccgaggcagctaagaaggcaatcgctgaatggggtcgtccagcagcagacatcacccacctggtggtcaccaccaactccggcgctcacgtgccaggtgtcgatttccgtctggtgcctctgctgggtctgcgtccatccgtccgtcgcaccatgctgcacctgaacggttgcttcgctggttgcgctgcactgcgtctggcaaaggacctggctgagaactcccgcggcgcacgtgtcctggttgtggcagctgaactgaccctgatgtacttcaccggcccagatgagggttgcttccgcaccctgctggtgcagggtctgttcggtgatggtgcagcagctgtcatcgttggtgccgatgcagatgacgtcgaacgcccactgttcgagatcgtttccgccgcacagaccatcatcccagaatccgaccacgctctgaacatgcgtttcaccgagcgccgcctggatggtgttctgggtcgtcaggtgccaggtctgatcggtgacaacgtggaacgctgcctgctggatatgttcggtccactgctgggcggtgacggcggtggcggttggaacgacctgttctgggcagtccacccaggttcctccaccatcatggatcaggttgatgctgcactgggtctggagccaggcaagctggcagcttcccgtcgcgtgctgtccgactacggcaacatgtccggtgctaccgtcatcttcgccctggatgaactgcgtcgccagcgtaaggaagcagcagctgctggtgaatggccagagctgggtgttatgatggcattcggccctggtatgaccgtggacgcaatgctgctgcacgctacctctcacgtcaactaa

SEQ ID NO: 13 - DNA, 1170 bp, Curcuma longa
  source 1..1170: mol_type = other DNA
atggaagcgaacggctaccgcataactcacagcgccgacgggccggcgacgatcttggccatcggcaccgccaaccccaccaacgtcgtcgatcagaacgcttatcccgacttctatttccgggtcaccaactccgagtatctgcaggaactcaaagccaagtttaggcgcatctgtgagaaagcggccatcaggaagaggcacttgtacttgactgaggagattttgcgggagaatcctagcttgctggctcccatggcgccgtcgttcgacgcgcggcaggcgatcgtggtggaggcggtgccgaagctggcgaaggaggcggcggagaaggcgatcaaggagtggggccgccccaaatcggacatcacgcacctcgtcttctgctccgcgagcggaatcgacatgcccggctccgacctgcagcttctcaagctgctcgggctcccgccgagcgtcaatcgcgtcatgctctacaacgtcgggtgccacgccggtggcaccgccctccgcgtcgccaaggacctcgcggagaacaaccgcggcgcgcgggtgctcgccgtctgctccgaggtcaccgtgctctcctaccgcggcccccaccccgcccacatcgagagcctcttcgtccaagctctgtttggcgacggcgccgccgcgctcgtggtcgggtccgaccccgtcgatggcgtcgagcgccccatcttcgaaatcgcctcggcatcccaagtgatgcttccggagagcgcagaggcggtgggcggccacctccgcgaaattgggctgaccttccacctcaagagccagcttccgtcgatcatcgcgagcaacatcgagcagagcctgacgactgcgtgctcgccgctggggctgtcggactggaaccagctgttctgggcggttcaccccggcggccgagcgatcctggaccaggtggaggcgcggctcggactggagaaggaccggctcgccgcgacgcggcacgtactcagcgagtacggcaacatgcagagcgccacggtgctgttcatcctggacgagatgcggaaccgctcggctgcggagggccacgccaccaccggcgaggggctcgactggggcgtgctgttgggcttcggcccgggactctccatcgagaccgtcgtcctccatagttgcagactgaactag

SEQ ID NO: 14 - DNA, 1170 bp, synthetic construct
  source 1..1170: mol_type = other DNA
atggaagcaaacggctaccgcatcacccactccgctgatggtccagccaccatcctggcaatcggcaccgctaacccaaccaacgtggtcgatcagaacgcctacccagacttctacttccgcgtcaccaactccgaatacctgcaggagctgaaggctaagttccgccgcatctgcgaaaaggcagctatccgcaagcgccacctgtacctgaccgaagagatcctgcgcgagaacccatccctgctggcaccaatggctccatccttcgatgcccgccaggcaatcgttgtggaagccgtgccaaagctggcaaaggaagccgcagagaaggcaatcaaggagtggggccgcccaaagtccgacatcacccacctggtcttctgctccgcttccggtatcgatatgccaggctccgacctgcagctgctgaagctgctgggtctgccaccatccgtcaaccgcgttatgctctacaacgttggttgccacgccggcggtaccgcactgcgcgtcgctaaggatctggccgaaaacaaccgcggtgcacgtgtgctggctgtctgctccgaggttaccgtgctgtcctaccgtggtccacacccagctcacatcgaatccctgttcgtgcaggcactgttcggtgatggtgctgcagcactggtcgttggttccgatccagttgacggcgtggaacgcccaatcttcgagatcgcctccgcatcccaggtcatgctgccagaatccgctgaggctgttggcggtcacctgcgcgaaatcggtctgaccttccacctgaagtcccagctgccatccatcatcgcatccaacatcgagcagtccctcaccaccgcttgctccccactgggtctgtccgactggaaccagctgttctgggctgttcacccaggcggtcgtgcaatcctggatcaggtggaagcacgcctgggtctggagaaggaccgtctggctgcaacccgtcacgtcctgtccgaatacggcaacatgcagtccgcaaccgttctgttcatcctggatgagatgcgcaaccgctccgcagctgaaggtcacgctaccaccggtgaaggtctggactggggcgtgctgctgggtttcggtccaggtctgtccatcgagaccgtggtcctgcactcctgccgcctgaactaa

SEQ ID NO: 15 - DNA, 1170 bp, Curcuma longa
  source 1..1170: mol_type = other DNA
atggccaacctccacgcgttgcgcagggagcagagggctcaaggtcccgccaccatcatggccatcgggacggccacccctcccaacctctacgagcagagcaccttcccggacttctacttccgcgtcaccaactccgacgacaagcaggagctcaagaaaaagttccgccgcatgtgcgagaagacaatggtgaagaagcggtacctgcacttgaccgaggagatcctgaaggagaggcccaagctctgctcctacaaggaggcgtcgttcgacgaccggcaggacatcgtggtggaggagataccgagattggctaaggaagctgcggagaaggccatcaaggagtgggggcggcccaaatcggagatcacccacctggtcttctgttccatcagcggcatcgacatgcccggcgccgactaccgcctcgcgacgctcctcggcctccctctcaccgtcaaccgcctcatgatctacagccaggcctgccacatgggcgccgccatgctccgcatcgccaaggacctcgccgagaacaacaggggcgcgcgcgtgctggtggtcgcctgcgagatcaccgtgctcagcttccgcggcccgaacgagggtgacttcgaggcgctcgcggggcaggccggcttcggcgacggcgcgggggccgtcgtcgtcggggccgacccgctggaaggaattgaaaaacccatctacgagatcgcggcggcgatgcaggagacggtggcggagagccagggggcggtgggcggccacctgcgggcgttcggctggacgttctacttcctgaaccagctgccggcgatcatcgccgacaacctcgggaggagcctggagcgggcgttggcgccgctgggggtgagggagtggaacgacgtcttctgggtggcgcacccgggcaactgggccatcatggacgccatcgaagccaagctgcagctgagcccggacaagctcagcaccgcccgccacgtcttcacagagtacggcaacatgcagagcgccaccgtgtacttcgtgatggatgagctgaggaagcggtcggcggtggaggggcggagcaccaccggagacggcttgcagtggggagttctcctcggttttgggccgggcctcagcatcgagaccgttgtactgcgcagtatgccactgtag

SEQ ID NO: 16 - DNA, 1170 bp, synthetic construct
  source 1..1170: mol_type = other DNA
atggccaacctgcacgcactgcgtcgcgaacagcgtgctcagggtccagcaaccatcatggcaatcggcaccgctaccccaccaaacctgtacgagcagtccaccttcccagatttctacttccgcgtcaccaactccgatgacaagcaggaactgaagaagaagttccgtcgcatgtgcgagaagaccatggttaagaagcgctacctgcacctgaccgaagagatcctgaaggaacgcccaaagctgtgctcctacaaggaagcatccttcgatgaccgccaggacatcgtggtcgaagagatcccacgcctggcaaaggaagcagctgagaaggctatcaaggaatggggccgcccaaagtccgagatcacccacctggtgttctgctccatctccggtatcgatatgccaggtgctgattaccgtctggcaaccctgctgggtctgccactgaccgtcaaccgcctgatgatctactcccaggcatgccacatgggtgccgcaatgctgcgcatcgccaaggatctggcagaaaacaaccgcggcgcacgtgtgctggttgtggcatgcgagatcaccgtcctgtccttccgcggtccaaacgaaggcgacttcgaggctctggctggtcaggctggtttcggtgatggcgcaggtgctgtcgttgtgggtgcagacccactggaaggcatcgagaagccaatctacgaaatcgctgccgcaatgcaggaaaccgtcgcagagtcccagggtgctgttggcggtcacctgcgcgctttcggttggaccttctacttcctgaaccagctgccagctatcatcgccgataacctcggtcgctccctcgaacgtgcactggcaccactgggcgttcgtgagtggaacgacgtgttctgggtcgctcaccctggtaactgggccatcatggatgcaatcgaagctaagctgcagctgtccccagacaagctgtccaccgctcgccacgtgttcaccgagtacggcaacatgcagtccgccaccgtttacttcgtgatggatgaactgcgcaagcgctccgcagttgaaggtcgctccaccaccggtgatggtctgcagtggggcgtgctgctgggtttcggtccaggtctgtccatcgagaccgtcgttctgcgctccatgccactgtaa

SEQ ID NO: 17 - DNA, 1176 bp, Curcuma longa
  source 1..1176: mol_type = other DNA
atggcgatgatcagcttgcaggcgatgcgcaaggcgcagagagctcaaggtccggccaccatcttggccgtcggcaccgccaacccgcccaatctctacgagcaggacacgtatcccgactactacttccgcgtcaccaactccgagcacaagcaggagctcaagaacaagttccgcctcatgtgcgagaagacgatggtgaagaggcggtatctttacctgacgccggagatcctgaaggagcggccgaagctgtgctcgtacatggagccgtcgttcgacgaccggcaggacatcgtggtggaggaggtgccgaagctggccgcggaggcagcggagaacgccatcaaggagtggggcggcgacaagtccgccatcacccacctggtcttctgctccatcagcggcatcgacatgcccggagctgactaccgcctcgcccagctcctcggactcccgctcgccgtcaaccgcctgatgctctacagccaggcctgccacatgggcgccgccatgctgcgcatagccaaggacatcgccgagaacaaccgctccgcgcgcgtcctcgtcgtcgcctgcgagatcaccgtgctcagcttccgcggcccggacgagcgcgacttccaggcgctggccggccaggccggcttcggggacggcgccggcgcgatgatcgtcggggccgaccccgtcctcggcgtcgagcggccgctctaccacatcatgtcggcgactcagacgacggtaccggagagcgagaaggcggtggggggccacctccgcgaggtggggctgaccttccacttcttcaaccagctgccggcgatcatcgccgacaacgtggggaacagcctggcggaggcgttcgaaccgatcgggatcaaggactggaacaacatcttctgggtggcgcacccgggcaactgggccatcatggacgccatcgagaccaagctgggcctggaacagagcaagctggccaccgcacgccacgtcttctccgagttcggcaacatgcagagcgccaccgtctacttcgtgatggacgagctcaggaaacggtcggcggcggagaaccgggcgaccaccggcgacgggctccggtggggcgtgctcttcggcttcggcccgggcatcagcatcgaaaccgtcgtgctccaaagcgtgccgctttag

SEQ ID NO: 18 - DNA, 1521 bp, Curcuma longa
  source 1..1521: mol_type = other DNA
atgaatacaattaacgaatatttaagtttagaagaatttgaggccataatctttggaaatcaaaaagttacaattagcgacgttgtcgtaaaccgagttaatgaaagtttcaatttcttaaaagaattctctgggaataaagtaatttacggcgtaaacactggttttggaccaatggcgcagtatagaattaaagagtctgatcaaattcagcttcaatataatttaattagaagccactcttcgggaaccggaaagccattaagcccggtttgtgctaaagcagcaattttagctcgtttaaacactctttcattaggaaattcaggcgttcacccgtcagtaatcaacctaatgtctgagcttatcaataaagatattacccctttaatcttcgaacacggaggcgttggtgccagcggtgacttagtacagctgtcacatttagctttagtgttaattggcgaaggtgaagttttttataaaggtgaaagaagaccaactcctgaagtttttgaaattgaaggtttaaaaccaattcaggtagaaattagagaaggtctggcattaattaacggaacttcagtaatgactggaattggagttgtaaatgtttatcatgctaaaaaattattagactggtcattaaaatcttcttgtgcaattaacgaattggttcaggcttatgacgatcatttctcagcagaactaaaccagactaaacgtcataaaggacagcaggaaattgcgttgaaaatgcgtcaaaatctttcagacagtactttaatccgtaaaagagaagatcatttatattctggtgaaaataccgaagaaatcttcaaagaaaaagttcaggaatattattcattaagatgcgttcctcaaattttaggaccggttttagaaactattaataatgtagcttctattctggaagacgaatttaactcggcaaacgataacccaattatcgatgtaaaaaaccagcatgtttaccacggcggaaatttccacggagattatatttcgcttgaaatggataaactaaaaattgttattaccaaattaacaatgctggcagaacgtcagttgaactatttattaaattcaaaaatcaacgaattacttcctccgtttgtaaacttaggaacattaggatttaatttcggaatgcagggtgttcagtttacagcaacatctacaacggcagaaagtcaaatgctgtcgaacccaatgtatgttcacagtattccaaacaacaacgacaatcaggatatcgtaagtatgggaactaactcggcagtaattacctcaaaagtaatcgaaaatgcttttgaagttctggctatcgaaatgattactatcgttcaggcaattgattatttaggacaaaaagacaaaatttcatctgtttctaaaaaatggtacgatgaaattagaaatataattccaacatttaaggaagatcaggtaatgtatcctttcgttcaaaaagtaaaagatcatttgatcaacaattaa

SEQ ID NO: 19 - DNA, 1686 bp, Arabidopsis thaliana
  source 1..1686: mol_type = other DNA
atggcgccacaagaacaagcagtttctcaggtgatggagaaacagagcaacaacaacaacagtgacgtcattttccgatcaaagttaccggatatttacatcccgaaccacctatctctccacgactacatcttccaaaacatctccgaattcgccactaagccttgcctaatcaacggaccaaccggccacgtgtacacttactccgacgtccacgtcatctcccgccaaatcgccgccaattttcacaaactcggcgttaaccaaaacgacgtcgtcatgctcctcctcccaaactgtcccgaattcgtcctctctttcctcgccgcctccttccgcggcgcaaccgccaccgccgcaaaccctttcttcactccggcggagatagctaaacaagccaaagcctccaacaccaaactcataatcaccgaagctcgttacgtcgacaaaatcaaaccacttcaaaacgacgacggagtagtcatcgtctgcatcgacgacaacgaatccgtgccaatccctgaaggctgcctccgcttcaccgagttgactcagtcgacaaccgaggcatcagaagtcatcgactcggtggagatttcaccggacgacgtggtggcactaccttactcctctggcacgacgggattaccaaaaggagtgatgctgactcacaagggactagtcacgagcgttgctcagcaagtcgacggcgagaacccgaatctttatttccacagcgatgacgtcatactctgtgttttgcccatgtttcatatctacgctttgaactcgatcatgttgtgtggtcttagagttggtgcggcgattctgataatgccgaagtttgagatcaatctgctattggagctgatccagaggtgtaaagtgacggtggctccgatggttccgccgattgtgttggccattgcgaagtcttcggagacggagaagtatgatttgagctcgataagagtggtgaaatctggtgctgctcctcttggtaaagaacttgaagatgccgttaatgccaagtttcctaatgccaaactcggtcagggatacggaatgacggaagcaggtccagtgctagcaatgtcgttaggttttgcaaaggaaccttttccggttaagtcaggagcttgtggtactgttgtaagaaatgctgagatgaaaatagttgatccagacaccggagattctctttcgaggaatcaacccggtgagatttgtattcgtggtcaccagatcatgaaaggttacctcaacaatccggcagctacagcagagaccattgataaagacggttggcttcatactggagatattggattgatcgatgacgatgacgagcttttcatcgttgatcgattgaaagaacttatcaagtataaaggttttcaggtagctccggctgagctagaggctttgctcatcggtcatcctgacattactgatgttgctgttgtcgcaatgaaagaagaagcagctggtgaagttcctgttgcatttgtggtgaaatcgaaggattcggagttatcagaagatgatgtgaagcaattcgtgtcgaaacaggttgtgttttacaagagaatcaacaaagtgttcttcactgaatccattcctaaagctccatcagggaagatattgaggaaagatctgagggcaaaactagcaaatggattgtga

SEQ ID NO: 20 - DNA, 1686 bp, synthetic construct
  source 1..1686: mol_type = other DNA
atggcaccacaggaacaggctgtctcccaggttatggagaagcagtccaacaacaacaactccgatgttatcttccgctccaagctgccagacatctacatcccaaaccacctgtccctgcacgattacatcttccagaacatctccgaattcgcaaccaagccatgcctgatcaacggtccaaccggccacgtgtacacctactccgatgtccacgttatctcccgccagatcgcagctaacttccacaagctgggcgtgaaccagaacgacgtggtcatgctgctgctgccaaactgcccagagttcgtcctgtccttcctggctgcatccttccgcggtgccaccgcaaccgctgcaaacccattcttcaccccagctgaaatcgccaagcaggctaaggcctccaacaccaagctgatcatcaccgaggctcgctacgttgacaagatcaagccactgcagaacgatgacggcgttgtgatcgtctgcatcgatgacaacgaatccgttccaatcccagagggttgcctgcgcttcaccgaactgacccagtccaccaccgaagcatccgaggttatcgattccgtggagatctccccagatgacgtcgttgctctgccatactcctccggtaccaccggtctgccaaagggcgtcatgctgacccacaagggtctggtgacctctgtggcacagcaggttgacggcgaaaacccaaacctgtacttccactccgatgacgtcatcctgtgcgttctgccaatgttccacatctacgctctgaactccatcatgctgtgcggtctgcgtgttggtgcagctatcctgatcatgccaaagttcgaaatcaacctgctgctggagctgatccagcgctgcaaggtgaccgtcgcaccaatggtgccaccaatcgtcctggcaatcgctaagtcctccgaaaccgagaagtacgatctgtcctccatccgcgtggtcaagtccggtgccgcaccactgggcaaggaactggaggacgcagtgaacgctaagttcccaaacgccaagctgggccagggttacggtatgaccgaagctggtccagtgctggcaatgtccctgggtttcgcaaaggagccattcccagtcaagtccggtgcttgcggcaccgttgtgcgcaacgccgaaatgaagatcgtcgatccagacaccggcgattccctgtcccgcaaccagccaggcgagatctgcatccgcggccaccagatcatgaagggttacctgaacaacccagctgccaccgcagagaccatcgataaggacggctggctgcacaccggtgacatcggcctgatcgatgacgatgacgaactgttcatcgttgaccgcctgaaggagctgatcaagtacaagggcttccaggtggccccagcagaactggaggctctgctgatcggtcacccagacatcaccgacgtcgccgtcgttgcaatgaaggaagaggcagctggcgaagttccagtggccttcgtggtcaagtccaaggattccgaactgtccgaggatgacgttaagcagttcgtgtccaagcaggttgtgttctacaagcgcatcaacaaggttttcttcaccgagtccatcccaaaggctccatccggcaagatcctgcgcaaggacctgcgcgctaagctggccaacggtctgtaa

SEQ ID NO: 21 - DNA, 936 bp, Corynebacterium sp.
  source 1..936: mol_type = other DNA
atgtctctcaatggaaaagtcgccatcgttaccggatctggtgcaggacttggtcgttccttcgctcaggagcttgcccgtcagggtgcatctgtcatcgtcaatgacgtaaaccaggcagccgcagatgagactgtcgcagcaatcaccgaagccggcggcaaagccgccgccgttatcgcccccgttggaccctctgaaagcgccgcattgctggtgcgggaggccgtcgacaagttcggttctttggacattcttgtcacaaacgcgggcatccttcgtgataggtccctgctgaagatgacggacgatgatttcgatgcagtcattaacgtgcacctcaagggcactttcacctgtgttcgcgaggcatttggatacttcaaggagaatggaatcgcggggcgcatcgtcacgattggttctcccaccgggcagcgcggcaacttcggacagagcaattacgctgcagctaaggcgggcattgtgggtatggttcgcacgtgggcgctggagatgaagcgcgcaggtgtcaccattaacgcgatcattccggaagcagccaccgatatgaccaagacggtgccatatttccagaaggctgtagaggccgatgagcgtggcgaggccatgccagcattcttccgcgagaccctaggttttggcactcctcaggatgttgcgggacttgtggccttcctttcctctgatgaggcagcgaatatttctggacaggccatcggtgcaggcggcgaccgcatgcaggtgtggaagcacccagagccagcagttactgaatttaacccaggtggctggacctatgaagcactgcaggaacgtggcaagaacattattgagggcaacctgcagtccgtcggtgtcgttttccctgaactgccggcagagcttcagccacaaatcccagtcaaggcataa

SEQ ID NO: 22 - DNA, 945 bp, Corynebacterium sp.
  source 1..945: mol_type = other DNA
atgagcaacaacgtagtgaaatatgagtgcgcggtcgacgccgacaacattgtcgcagtcgatatgcatgtgcacttggaagtcgacagctgcggacacaaatcgatgccggcagacatcatggcggcatcctcgaagtactttaagaccgcggaacgaactccctcagcagatgccattgctgatatttatagggaacacaagatggcggcggtggttttcaccatcgatgcgcggacccaaatggggcatctgccgaactcgattgatgatttggtggcaagctgtgcccgcaacaatgacgtgctgatcccttttggcagtgtggatcctcgtaccggcgaggacgcgctggtggaagctcgccgacaggtggaagaactcggggtgcgaggcttcaaattccatccatcggttcaaggattcgacccatccgcgccagagttctacccactgtgggaattgctcgaaagttttggattgccatgcgtgttccataccggacaaaacggcatgggtgcaggtcttccaggtggtcgaggcattaagctgcgcttctccaacccaatgttgcttgatgatgttgcggcggacttcccgaacctgaccatcatcatggcgcacccttctgttccttggcaggatgaggctaactcgattgccacccacaaggccaatgtgttcattgatctttccggctggtcgccgaagtatttcccagagtctttggtcagacagtccaataacgtgctatccaagaaggtgctgtttggcacggacttcccgctgattaccccagagaaatggcttgcggctttcgcgaatctgccactgaaggatgaggttcgtccgggaatcctcaaagacaatgcggtgaaggtacttggcctagccgctagcactgagcgcggatctcaagcagaaaaggtcgtgcaacatgcgtga

SEQ ID NO: 23 - DNA, 1197 bp, Corynebacterium sp.
  source 1..1197: mol_type = other DNA
atgcgtgatcccattcaaggtgctgttattccttctgatctttttggtttcgcagaagttctcaccgaagccgaacgcgcagttcttctggaaacccgcagggtgcttgaggaagaggtgaagccttatattaatgaggcctgggataaggcagtcttccccgatgagatcgtgcagcccctccaagatctgcaattgcttgatccgcctgcacttcgggaagcaggggagtcggttcgagacattttcactggtttccgcaattttgaactcgcgcgctgtgacatcaatgttggtacctattacaacgcatctgctggtctcttccgaacggcctgcatggttggtggctccccggagcaggcgcagcgattggatgcgcagatcaaatctggtgaggtcaagggcgtttttgcactgacggaacctgatcatggctctgatatcgcaggtggtctggcaaccacggccactaaggacgcagacaccggcgagtggattatcaatggtgaaaaacggtggatcggtggtgcttccactgctgatttgatcgctaccttcgccagggatacagccgataaccaggtgaaatgcttcctcgtggcacctcaggcagagggcgtgtccatggagattattgatcgcaaagcctcactgcgcatcatgcaaaatgcacacattacctataacaatgtccgggtgtctggggatgcgcggctgcacaacatcaattctttcaaggatgtttcggaatgcctgcgccgtatgcgttccgatgtggcgtggatggcggtcggtgcgcaggcaggtgcctatgaagcagccgtgaagtatgtgcgcagcagggaacagtttggccgtccgatcgcggggttccagttgattcaggaaaagctcgcgctcatgctgggcaatctcacggcgtcgctgggcatgatggtcaaactcaccgatcagcagcaggcgggaattttcaaagaggaaaactccgcgctggcgaaaatgtttacctcgctcaaacttcgggagaccgctagttgggcgcgggaaatctgcggaggcaacggcatcattttggacaacgatgttgcccggttccatgccgatgcagaagccgtctattcatatgaaggcacccacgaaatcaatgcactcatcgttggtcgcgccatcacgggcgtcagcgcttttatctaa

SEQ ID NO: 24 - DNA, 474 bp, Corynebacterium sp.
  source 1..474: mol_type = other DNA
atgactacttccaccaccccaaacaccatcgtttctttcgaagacgcaccaaccctcaccggccaggacctgggcttttcgcagtggcgcactgtcacccaggagatggtgaacaccttcgcggacgcaactgatgatcagcagtggattcacactgatcctgagcgcgccaaggacggtccttttggtggcgcaattgcccacggtttcctcaccttgtccatgatcattccgttctggggcgagcttctcgatgtcaccggcgtgaccaccaaggtgaactatggcctggataaggtgcgtttcacctctcccgtcaaggtcggttcccgcatccgcatgggcgctgtggtccgtgagatctctgaggtgaagggcaatggcctgcacctggtcgccgatggcactattgagatcgaagggcaggagcgcccggccgtcgtagctaccttcctcacccgcttctacgcttaa

SEQ ID NO: 25 - DNA, 468 bp, Corynebacterium sp.
  source 1..468: mol_type = other DNA
atgaccaccagcaaccccaccgccgagatcattggcggaccagaacgattcctcgaggccgaattgtcccagcagattcaattcctcactgcccgcgcacgagccaagggatccgccaaaggaaacgaagccttagtcgacctcggacttaaagttcgccaatactccacactgtccctagcggccagcggattaaaaccaacccaacgagaattgggagcatttctcgacctagacccaagtcagattgttgccttggtcgatttcctagaaaagcgcggattagtggcccgggaagttgacccccgggataggcgctcgaagatcatcatcgccaccgaaaaaggtctggaaattcacgacgaagccaccaaacgcctcctcatcgccgagggtgaatctctaaaaaacctcacctccgacgagcaagaacaactaagggaactgctgctcaaaatcgccttttaa

SEQ ID NO: 26 - DNA, 1539 bp, Corynebacterium sp.
  source 1..1539: mol_type = other DNA
atgaaagtgaacctcggaataggaagctacccacgacgcagggcaactgttcgaccagagtccactgcaatcgaattcgaaggcaccagcatcacctacggagaattcagcaaacgagtcaatcggcttggacatgctcttctagacctcggcgttgcgcaccaagatcgagtagcttatgtcggattcaaccaccctgccctgctagaagtgttcttttcaacgaacctcattggggcaacacccgtgcttgttaaccctcgcctatcggcaaacgaaatcgattacatcatccaagacagcggtgcgagcatcgtgttttacggaatcgacctcatcgagcacgccacttacctccaagaactccatccagagatcatcatggtggccgttgaaggcgatgagggtccaggtttgcgtcgaaaagcgcttattgaagcggcgagcgacgccgacatcgacctagaagtcagcgatgatgacatcgcgctgctcatgtacacctccggaaccactggccgcccaaagggcgccatgttatcccaccgaaacctcttctttaactacttcaatgccctgctcagccaggaaattgaacaaggcgcggtacttttatccactgcgccgttattccacatcgcgggcctcaacatgaccaccatcccggtgatgatgaagggcggaaaggtgatcatccaccgcgaattccgggcagagcacgtcctcgacgaaatcgaacgctccaaggtatccgaatccttcatggtgccagcgatgatcgacatgttgtccaaccacccatcatttgccgaacgcgacctttcttcccttcgcgccatcatggtgggcggctctccccttagcgaacgtgcgctgcgaatctggcaaggacgcgacgtaaaaattgtccaaggcttcggcatgacagaaaccgcaccgggcgcctgtatcctcgaggcaacagacacaagcacacaccttggaaccgcaggtcgagcccacttcttcaccgacatcaaactagtggacccgaaaaccggcgaagaagtccccaccggagaggccggcgaagttctcatccgcggaccacatgtgatgaccggatactggaaccgaccagaagacaccgccagcgcactacaaaatggctggtaccactccggagatatcgccatcaaagatgaagacggctactacaccatcaaagaccgcatcaaagacatgtacatctccggcggcgaaaacatttaccccgcagaagtcgaacaagcactccaggaactggaagcagtccttgatgccgcagtcatcggagtccccgatgaacgatggggcgaaactggcatcgcctttgtctccatccgagaaagctacctgaccaacccaccaaccggaccggaactacgagaactactaggcagtgtcctagccagatacaaacttccacgagaaatccacatcatcgaagaactcccccgcaacgccacaggcaaaatccaaaagaacatcctgcgagacttcaccatccccgtttcataa

SEQ ID NO: 27 - DNA, 1494 bp, Corynebacterium sp.
  source 1..1494: mol_type = other DNA
atgtccacaccagtttcaaatttggcaagcgttcagaaaactctggaccatgcgcttgaggaccgccctgaagagggaatcgtccgcgtcaaccgcaacatcttcactgaccctgagatcttcgagctggagatgcgccacatcttcgaaggcaactggatctacctggctcacgagtcccagatccctaacgctggcgactacttcaccacctacattggccgccagccgatcatgatcacccgttccaaggacggcacactcaactgcctgatcaacgcgtgttctcaccgtggcgccatgctctgccgtcgcaagactgacaaccgcaccaccttgacctgcccattccacggctggacattcagcaacgacggcgcactgctcaaggtcaaggacgaaaaagaaggcgcctacccagagaatttccgcaccgacggctcccacgatctgcgtcgcgttcctaagttcgagtcctaccgtggcttcctcttcggctccctcaacgatgatgtcgtttctttggaagagcacctcggcgacacccgtaccgtcattgacatgctggttgaccaatccccagaaggcctcgaagtactgcgcggatcctccacctacacctacgacggcaactggaagctccagaccgaaaacggtgcagacggctaccacgtttcctccacccactggaactacgctgcaaccacctcccgccgtggcactggtgaatccgcgaacgaaaccaaggcaatggacgctggtacctggggcaagcagggtggcggatacttctcctacccttacggccacatgctgctgtggatgtggtggggcaacccagaagaccgcccactgttcgagcgccgcgacgagttcaagaaggaattcggcgaagaaaagggcgagttcatggttggtgcttcccgcaatctgtgcctctaccccaatgtttacctgatggatcagttctcctcacagatccgccacatccgcccaatctcagttgatcagaccgaagtcaccatctactgcatcgcacctaagggcgagtccgcggaagcacgtgcaaaccgcatccgccagtacgaagacttcttcaacgcaacgggcatggcaaccccagatgacctggaggaattccgctcctgccagaagacctaccaggcatctgccttcccatggaatgacatgacccgcggtttgggccaccaggtacagggaccaaacgaggttgccaagggcctaggcatgaacgaagttctttcctccggagcacgcaccgaagatgaaggcctctacccaatccagcacggcttctggcatgaactcatgcaggaggctgtgaataagcagagcatcaaggaaaaggaattggctgacgataccgcttcttcccttgccaccgtagctgcagccaaaatccgtgaggaagcaaaggcagccgcgaagtccgacgctggagagcctcgccgccgtcgtcgcacccgcggttag

SEQ ID NO: 28 - DNA, 495 bp, Corynebacterium sp.
  source 1..495: mol_type = other DNA
atgtctgaaatcacccgctctgagatcgaagctttcctctactacgaggctcgcctgctcgatgaccgtaaatttgaagaatggctcgaatgctaccgcgaggacgccgagttttggatgccagcctgggacgacaacggtgaactgactgaagatccacagtctgaaatttccctcatctactacccaaaccgtggtggacttgaggaccgcgtcttccgcatccgcaccgaacgctcctctgcaacttccctacctgaaccacgcaccggccacagcaccaccaacgtggaaatcctggagcgccgcgacggcgaagtagatatccgcttcaactggatcaccttctactaccgttacaacaccaccgacacctacttcggcaccacgtttatcacccttgatgtcagtggtgaaaccccgaagatcgtcaagaagaaggtcgttttgaagaacgactacatccaccacatcgtcgatatttaccacgtctag

SEQ ID NO: 29 - DNA, 1539 bp, Corynebacterium sp.
  source 1..1539: mol_type = other DNA
atgactcaccaagttgcacttgcctttgaagacggcatcacccgattcatcgactgcgaagatgaccaaactgttgcagatgccgcctaccaggcacgcatcaacattcctttcgactgccgcgacggcgcctgcggaacctgcaaagcgttctgcgaatccggcgactttgacgaaggcgactacatcgacgacgccctgtccgaagatgaagcagccgacggctactgcctgccttgccagatgaccccaaagaccgacctcatcttgcagatcgccaccacctccgtgctggcaaagaccggcgcatccactttcgatggcgagttgaaggagatcaatcacttctctgattccaccatcggcattgagatcgaactggaaaaccgccaagatttggcgttcctccctggtcaatacatgaacatccaggttccaggcagcgaccagactcgttcctactctttctcctgcgctcaagattccggcaacgtgcagttcctgatcaaggtaaccccaggtggactcatgaccacctatctcaccgatcacgcgaaggtcggcgacaagctcaccttgaccggcccgatgggttccttcttcctgcgtgaacctgtccgcccgatcctgctgctcgccggcggaactggacttgcaccgatcttggctattttggaaaagctttcccgcgatgagcttctcgacgtcccaatccgcctggtttacggcgcgaacttcacccacgatctggtggaattggatcgacttgatgccttcaaggacaagttcgacttcgattacatcaccgtgctttccgacaaggacaccgagcatccacgcaagggctacgtcccagcacacctgaccggcgaatatgagccagatgaggacactgatgtgtacctctgcggccctcctccaatggtcgaggccgtgcgccaattcctgggcaccctggagcatcctccgctggacttttattacgagaagttcacttccgccgctgcccctgctgctggtaagccagagatcaccgtggagaccagcgaagttgcagaggatttcaacctggtcgaggtgtccactccaggcatgtcttccggcgaggtgcactcttctgcaacccagctgcaggcccgcatggctctggagctcggcgcgctggagcttgcgatcaacaaactcggcgagcgcgacatcgagcgattccgcaacttggccgacatcgcgaactccttcatcgacggcgataagtttatcgacgcggtgaagttcaccgaggccaacgccgatttccacgagttcctcttccgccgcgcaaacaacgaggcgctgcttgcggcgtaccagaacctccaggttgttcaagaaatgaacgcaacccttccaggcgccgagtggattgatccggcaattgccaccgagcacttggcgcttgtcgacgccgtctcccagaatgatctcgagaccgcgagaacaatcattcgtgaacacgcggagcacggcattgacactatggttaaggccctcgagaaatga

SEQ ID NO: 30 - DNA, 831 bp, Corynebacterium sp.
  source 1..831: mol_type = other DNA
atgagcgcgccagtaggacaaggcatcgaaggtcgccccactcacgtcaccccggaacgcttctttggccagggtgttgtggttaccggagcggctcaaggcatcggcatggcagtggcacaccgcatcgcatatgaggatggcaacctagtgttggtggaccgttccccgctggtgcatgaagttgccgaagagctgcgtaaagcaggcgccggaacggtggattctttcatcgccgatctggaaacctttgaaggcgcaactgatgctttggaatttgccgggcagaagttgaagaaccttgatgtggtgatcaacaacgttggtggcaccatctgggcgaagccttatcaggaatactctgaggaagagatccgcaaggaaatcaaccgaagcctcttccccaccttgtggatgtgccgggccgcgttgccaattctgatcggaaatggtggtggaacgatcgttaatgtgtcctccatcgcgaccggtggtatcaaccgtgttccttatgctgcagcaaagggtggcgtcaacggcattgtttctgccatggcccgcgaagctgcaccgcataatgtgcgcgtggtggcaacggctcccggtggcacgctcgctccggaacgtgccgtcaaacgaggccctgggccagagggcgaattggaagaaaagtggtatcagcaaatcgttgatcaaaccattgattccagtttgatgaagcgctacggcaccctagaggagcaggtcgcgccgatctgtttcctcgcttctgaggaagcttcctacatcactggatcagtcatgccagtcggtggaggcgaccagggataa

SEQ ID NO: 31 - DNA, 1314 bp, Corynebacterium sp.
  source 1..1314: mol_type = other DNA
atgtttgaaagggatatcgtggctactgataacaacaaggctgtcctgcactaccccggtggcgagttcgaaatggacatcatcgaggcttctgagggtaacaacggtgttgtcctgggcaagatgctgtctgagactggactgatcacttttgacccaggttatgtgagcactggctccaccgagtcgaagatcacctacatcgatggcgatgcgggaatcctgcgttaccgcggctatgacatcgctgatctggctgagaatgccaccttcaacgaggtttcttacctacttatcaacggtgagctaccaaccccagatgagcttcacaagtttaacgacgagattcgccaccacacccttctggacgaggacttcaagtcccagttcaacgtgttcccacgcgacgctcacccaatggcaaccttggcttcctcggttaacattttgtctacctactaccaggaccagctgaacccactcgatgaggcacagcttgataaggcaaccgttcgcctcatggcaaaggttccaatgctggctgcgtacgcacaccgcgcacgcaagggtgctccttacatgtacccagacaactccctcaatgcgcgtgagaacttcctgcgcatgatgttcggttacccaaccgagccatacgagatcgacccaatcatggtcaaggctctggacaagctgctcatcctgcacgctgaccacgagcagaactgctccacctccaccgttcgtatgatcggttccgcacaggccaacatgtttgtctccatcgctggtggcatcaacgctctgtccggcccactgcacggtggcgcaaaccaggctgttctggagatgctcgaagacatcaagagcaaccacggtggcgacgcaaccgagttcatgaacaaggtcaagaacaaggaagacggcgtccgcctcatgggcttcggacaccgcgtttacaagaactacgatccacgtgcagcaatcgtcaaggagaccgcacacgagatcctcgagcacctcggtggcgacgatcttctggatctggcaatcaagctggaagaaattgcactggctgatgattacttcatctcccgcaagctctacccgaacgtagacttctacaccggcctgatctaccgcgcaatgggcttcccaactgacttcttcaccgtattgttcgcaatcggtcgtctgccaggatggatcgctcactaccgcgagcagctcggtgcagcaggcaacaagatcaaccgcccacgccaggtctacaccggcaacgaatcccgcaagttggttcctcgcgaggagcgctaa